European Patent Application EP 4 393 506 A1, published July 3, 2024. Title: Pharmaceutical composition of anti-IL4R antibody and use thereof. Applicant: Chia Tai Tianqing Pharmaceutical Group Co., Ltd. Application EP 22860563.0, filed August 25, 2022. The sequence listing filed with the application follows.

SEQUENCE LISTING (24 sequences)

SEQ ID NO: 1 - protein, 5 aa, Mus sp.
TYGMS

SEQ ID NO: 2 - protein, 17 aa, Mus sp.
TINSNGGSTSYPDSVKG

SEQ ID NO: 3 - protein, 10 aa, Mus sp.
FFRFRNAMDY

SEQ ID NO: 4 - protein, 11 aa, Mus sp.
RTSENIYSYLA

SEQ ID NO: 5 - protein, 7 aa, Mus sp.
NAKTLAE

SEQ ID NO: 6 - protein, 10 aa, Mus sp.
QHYYGPPTWT

SEQ ID NO: 7 - protein, 119 aa, Mus sp.
EVQLVESGGGLVQPGGSLKLSCAASGFTFSTYGMSWVRQTPDKRLELVATINSNGGSTSYPDSVKGRFTISRDNAKNTLYLQMSSLKSEDTAMFYCARFFRFRNAMDYWGQGTSVTVSS

SEQ ID NO: 8 - protein, 119 aa, synthetic construct
  UNSURE 47: note = W or L
  UNSURE 49: note = S or A
  source 1..119: note = VH of huC2C1A1A1-V1 to huC2C1A1A1-V4 and huC2C1A1A1-V9 to huC2C1A1A1-V16
EVQLVESGGGLVQPGGSLRLSCAASGFTFSTYGMSWVRQAPGKGLVXVXTINSNGGSTSYPDSVKGRFTISRDNAKNTLYLQMNSLRAEDTAVYYCARFFRFRNAMDYWGQGTLVTVSS

SEQ ID NO: 9 - protein, 119 aa, synthetic construct
  source 1..119: note = VH of huC2C1A1A1-V5 to huC2C1A1A1-V8
EVQLVESGGGLVQPGGSLRLSCAASGFTFSTYGMSWVRQSPDKRLEWVSTINSNGGSTSYPDSVKGRFTISRDNAKNTLYLQMRSLRAEDTAVYYCARFFRFRNAMDYWGQGTLVTVSS

SEQ ID NO: 10 - protein, 108 aa, Mus sp.
DIQMTQSPASLSASVGETVTITCRTSENIYSYLAWYQQKQGKSPQFLVYNAKTLAEGVPSRFSGSGSGTQFSLNINSLQSEDFGSYYCQHYYGPPTWTFGGGTKLEIK

SEQ ID NO: 11 - protein, 108 aa, synthetic construct
  UNSURE 46: note = L or F
  UNSURE 48: note = I or V
  source 1..108: note = VL of huC2C1A1A1-V1, huC2C1A1A1-V3 to huC2C1A1A1-V5, huC2C1A1A1-V7 to huC2C1A1A1-V9, huC2C1A1A1-V11 to huC2C1A1A1-V13, huC2C1A1A1-V15 and huC2C1A1A1-V16
DIQMTQSPSSLSASVGDRVTITCRTSENIYSYLAWYQQKPGKAPKXLXYNAKTLAEGVPSRFSGSGSGTDFTLTISSLQPEDFATYYCQHYYGPPTWTFGQGTKVEIK

SEQ ID NO: 12 - protein, 108 aa, synthetic construct
  source 1..108: note = VL of huC2C1A1A1-V2, huC2C1A1A1-V6, huC2C1A1A1-V10 and huC2C1A1A1-V14
DIQMTQSPSSLSASVGQRVTITCRTSENIYSYLAWYQQKQGKPPRFLIYNAKTLAEGVPSRFSGSGSGTEFTLTITSLQAEDFGVYYCQHYYGPPTWTFGPGTKLEIK

SEQ ID NO: 13 - protein, 327 aa, synthetic construct
  source 1..327: note = Heavy chain constant region of chimeric and humanized antibodies
ASTKGPSVFPLAPCSRSTSESTAALGCLVKDYFPEPVTVSWNSGALTSGVHTFPAVLQSSGLYSLSSVVTVPSSSLGTKTYTCNVDHKPSNTKVDKRVESKYGPPCPPCPAPEFLGGPSVFLFPPKPKDTLMISRTPEVTCVVVDVSQEDPEVQFNWYVDGVEVHNAKTKPREEQFNSTYRVVSVLTVLHQDWLNGKEYKCKVSNKGLPSSIEKTISKAKGQPREPQVYTLPPSQEEMTKNQVSLTCLVKGFYPSDIAVEWESNGQPENNYKTTPPVLDSDGSFFLYSRLTVDKSRWQEGNVFSCSVMHEALHNHYTQKSLSLSLGK

SEQ ID NO: 14 - protein, 107 aa, synthetic construct [sequence omitted]

SEQ ID NO: 15 - protein, 242 aa, synthetic construct
  source 1..242: note = Human IL4Ra-his
MGWLCSGLLFPVSCLVLLQVASSGNMKVLQEPTCVSDYMSISTCEWKMNGPTNCSTELRLLYQLVFLLSEAHTCIPENNGGAGCVCHLLMDDVVSADNYTLDLWAGQQLLWKGSFKPSEHVKPRAPGNLTVHTNVSDTLLLTWSNPYPPDNYLYNHLTYAVNIWSENDPADFRIYNVTYLEPSLRIAASTLKSGISYRARVRAWAQCYNTTWSEWSPSTKWHNSYREPFEQHHHHHHHHHHH

SEQ ID NO: 16 - protein, 242 aa, synthetic construct
  source 1..242: note = Cal-IL4Ra-his
MGWLCSGLLFPVSYLVLLQVAGSGSMKVLQEPTCVSDYISLSTCEWKMGGPTNCSAELRLVYQLVFLISETNMCVPENNGAAGCVCHLFMEDMVGADNYTLDLWAGQQLLWKGSFKPSEHVKPKAPENLTVYTNVSETLLLTWSNPYPPDNYLYEKLTYAVNIWNENDPTDSRIYDVTYQEPTLRIAASTLKSGVSYRARVRAWAQSYNSTWSEWSPSTKWYNAYKEPFEKHHHHHHHHHHH

SEQ ID NO: 17 - DNA, 357 bp, synthetic construct
  source 1..357: mol_type = other DNA; note = VH of mouse C2C1A1A1
gaggtgcagctggtggagtctgggggaggcttagtgcagcctggagggtccctgaaactctcctgtgcagcctctggattcactttcagtacttatggcatgtcttgggttcgccagactccagacaagaggctggagttggtcgcaaccattaatagtaatggtggtagtaccagttatccagacagtgtgaagggccgattcaccatctccagagacaatgccaagaacaccctgtacctgcaaatgagcagtctgaagtctgaggacacagccatgttttactgtgcaagatttttccgctttaggaatgctatggactactggggtcaaggaacctcagtcaccgtctcctca

SEQ ID NO: 18 - DNA, 357 bp, synthetic construct
  source 1..357: mol_type = other DNA; note = VH of chimeric C2C1A1A1
gaggtgcagctggtggagagcggcggcggactggtgcagcctggaggatccctgaagctgtcctgcgccgcctccggcttcaccttctccacatacggcatgtcctgggtgagacagacccctgataagagactggagctggtggccaccatcaacagcaacggcggcagcaccagctaccccgacagcgtgaagggcagattcaccatctccagagacaacgccaagaacaccctgtacctgcagatgtccagcctgaagagcgaggatacagccatgttctactgtgccaggttctttaggttcagaaatgccatggactactggggccagggcacctccgtgacagtgagcagc

SEQ ID NO: 19 - DNA, 357 bp, synthetic construct
  source 1..357: mol_type = other DNA; note = VH of huC2C1A1A1-V13 to huC2C1A1A1-V16
gaggtgcagctggtggagtccggaggaggactggtgcagcccggcggctctctgagactgagctgcgctgcctccggcttcacctttagcacctacggcatgagctgggtgagacaagcccccggcaaaggactggtgtgggtggctaccatcaacagcaacggcggctccacaagctaccccgacagcgtgaagggaagattcaccatctctagagacaacgccaagaacacactgtatctgcagatgaactctctgagagccgaagacaccgctgtgtactactgcgctagattctttagatttagaaacgccatggactactggggccaaggcacactggtgacagtgtcctcc

SEQ ID NO: 20 - DNA, 324 bp, synthetic construct
  source 1..324: mol_type = other DNA; note = VL of mouse C2C1A1A1
gacatccagatgactcagtctccagcctccctatctgcatctgtgggagaaactgtcaccatcacatgtcgaacaagtgagaatatttacagttatttagcatggtatcagcagaaacagggaaaatctcctcagttcctggtctataatgcaaaaaccttagcagaaggtgtgccatcaaggttcagtggcagtggatcaggcacacagttttctctgaatatcaacagcctgcagtctgaagattttgggagttattactgtcaacattattatggtcctcccacgtggacgttcggtggaggcaccaagctggaaatcaaa

SEQ ID NO: 21 - DNA, 324 bp, synthetic construct
  source 1..324: mol_type = other DNA; note = VL of chimeric C2C1A1A1
gacatccagatgacacagagccccgccagcctgtccgcctccgttggagagaccgtgaccatcacctgtaggacctccgagaatatctacagctacctggcctggtatcaacagaagcagggcaagtcccctcagtttctggtgtacaacgccaagaccctggccgagggcgtgccctctaggttctccggctccggcagcggcacccagttcagcctgaatatcaacagcctgcagagcgaggactttggcagctactactgtcagcactactacggccctcccacctggacatttggcggcggcacaaagctggagatcaag

SEQ ID NO: 22 - DNA, 324 bp, synthetic construct
  source 1..324: mol_type = other DNA; note = VL of huC2C1A1A1-V3, huC2C1A1A1-V7, huC2C1A1A1-V11 and huC2C1A1A1-V15
gacatccagatgacccagagccctagctctctgagcgcttccgtgggagatagagtgaccatcacatgcagaacctccgagaacatctacagctatctggcttggtatcagcagaagcccggcaaggcccccaagttcctggtgtacaacgccaagacactggctgagggcgtgcctagcagattcagcggctccggcagcggcacagactttacactgacaatcagctctctgcaacccgaggacttcgccacctactactgccagcactactatggcccccctacatggacctttggccaaggcaccaaggtggagatcaag

SEQ ID NO: 23 - DNA, 984 bp, synthetic construct
  source 1..984: mol_type = other DNA; note = Heavy chain constant region of chimeric and humanized antibodies
gccagcacaaagggcccttccgtgtttcccctggccccctgcagcaggagcacctctgagtccaccgccgccctgggctgtctggtgaaggactactttcccgagcccgtgaccgtgagctggaattccggcgccctgacatccggcgtgcacaccttccccgccgtgctgcagtcctccggcctgtacagcctgagctccgtggtgacagtgccttcctcctccctgggcaccaagacctacacatgtaatgtggatcacaagcccagcaacacaaaggtggataagagagtggagtccaagtacggccctccttgccctccctgtcctgccccagagttcctgggcggcccctctgtgttcctgttcccccctaagcccaaggacacactgatgatctccaggacccctgaggtgacctgcgtggtggtggacgtgagccaggaggaccctgaggtgcagttcaattggtacgtggatggcgtggaggtgcacaatgccaagacaaagcccagagaggagcagtttaattccacatacagggtggtgtccgtgctgaccgtgctgcaccaggattggctgaacggcaaggagtacaagtgtaaggtgagcaacaagggcctgccttcctccatcgagaagacaatcagcaaggccaagggccagcctagggagccccaggtgtacacactgcctcccagccaggaggagatgaccaagaaccaggtgagcctgacctgcctggtgaagggcttctaccctagcgacatcgccgtggagtgggagtccaacggccagcccgagaataactacaagacaacaccccccgtgctggattccgatggcagcttctttctgtactccaggctgaccgtggataagagcaggtggcaggagggcaatgtgttcagctgctccgtgatgcacgaggccctgcacaatcactacacccagaagagcctgtccctgagcctgggcaagtga

SEQ ID NO: 24 - DNA, 324 bp, synthetic construct
  source 1..324: mol_type = other DNA; note = Light chain constant region of chimeric and humanized antibodies
cgtacggtggcggcgccatctgtcttcatcttcccgccatctgatgagcagttgaaatctggaactgcctctgttgtgtgcctgctgaataacttctatcccagagaggccaaagtacagtggaaggtggataacgccctccaatcgggtaactcccaggagagtgtcacagagcaggacagcaaggacagcacctacagcctcagcagcaccctgacgctgagcaaagcagactacgagaaacacaaagtctacgcctgcgaagtcacccatcagggcctgagctcgcccgtcacaaagagcttcaacaggggagagtgttga